European Patent Application EP 4 748 944 A1, published May 27, 2026. Title: METHOD FOR PRODUCING CIRCULAR DNA. Applicant: Moderna Enzymatics Co., Ltd. The sequence listing filed with the application follows.

SEQUENCE LISTING (116 sequences)

SEQ ID NO: 1 - DNA, 18 bp, synthetic construct
  source 1..18: mol_type = other DNA
agtatgttgtaactaaag

SEQ ID NO: 2 - DNA, 264 bp, synthetic construct
  source 1..264: mol_type = other DNA
tattaaaaagaagatctatttatttagagatctgttctattgtgatctcttattaggatcgcactgccctgtggataacaaggatccggcttttaagatcaacaacctggaaaggatcattaactgtgaatgatcggtgatcctggaccgtataagctgggatcagaatgaggggttatacacaactcaaaaactgaacaacagttgttctttggataactaccggttgatccaagcttcctgacagagttatccacagtagat

SEQ ID NO: 3 - DNA, 300 bp, synthetic construct
  source 1..300: mol_type = other DNA
agtatgttgtaactaaagtattaaaaagaagatctatttatttagagatctgttctattgtgatctcttattaggatcgcactgccctgtggataacaaggatccggcttttaagatcaacaacctggaaaggatcattaactgtgaatgatcggtgatcctggaccgtataagctgggatcagaatgaggggttatacacaactcaaaaactgaacaacagttgttctttggataactaccggttgatccaagcttcctgacagagttatccacagtagatctttagttacaacatact

SEQ ID NO: 4 - DNA, 286 bp, synthetic construct
  source 1..286: mol_type = other DNA
ggatcctgggtattaaaaagaagatctatttatttagagatctgttctattgtgatctcttattaggatcgcactgccctgtggataacaaggatccggcttttaagatcaacaacctggaaaggatcattaactgtgaatgatcggtgatcctggaccgtataagctgggatcagaatgaggggttatacacaactcaaaaactgaacaacagttgttctttggataactaccggttgatccaagcttcctgacagagttatccacagtagatcgcacgatctgt

SEQ ID NO: 5 - DNA, 18 bp, synthetic construct
  source 1..18: mol_type = other DNA
agtatgttgtacctaaag

SEQ ID NO: 6 - DNA, 36 bp, synthetic construct
  source 1..36: mol_type = other DNA
gagctgttgacagagggtcattttcacactataatg

SEQ ID NO: 7 - DNA, 30 bp, synthetic construct
  source 1..30: mol_type = other DNA
tacagcctcctttcggaggctgttttttta

SEQ ID NO: 8 - DNA, 426 bp, synthetic construct
  source 1..426: mol_type = other DNA
gagctgttgacagagggtcattttcacactataatgcagtgaatcccaaacagtatgttgtacctaaagggatcctgggtattaaaaagaagatctatttatttagagatctgttctattgtgatctcttattaggatcgcactgccctgtggataacaaggatccggcttttaagatcaacaacctggaaaggatcattaactgtgaatgatcggtgatcctggaccgtataagctgggatcagaatgaggggttatacacaactcaaaaactgaacaacagttgttctttggataactaccggttgatccaagcttcctgacagagttatccacagtagatcgcacgatctgtcagctcatttcctttaggtacaacatactagaatatttgcctacagcctcctttcggaggctgttttttta

SEQ ID NO: 9 - DNA, 149 bp, synthetic construct
  source 1..149: mol_type = other DNA
tttttgatgccatcagaaaacgcgtcagcgccgctctgaggcaataaacagaatcaggcataaaatcagccgcacagattttttaaaacgcgccacgggatttttaaaccggtatttaacggtgtatgaatcccgttttatcttccttt

SEQ ID NO: 10 - DNA, 582 bp, synthetic construct
  source 1..582: mol_type = other DNA
gagctgttgacagagggtcattttcacactataatgcagtgaatcccaaacagtatgttgtacctaaagggacctgtttttgatgccatcagaaaacgcgtcagcgccgctctgaggcaataaacagaatcaggcataaaatcagccgcacagattttttaaaacgcgccacgggatttttaaaccggtatttaacggtgtatgaatcccgttttatcttcctttggatcctgggtattaaaaagaagatctatttatttagagatctgttctattgtgatctcttattaggatcgcactgccctgtggataacaaggatccggcttttaagatcaacaacctggaaaggatcattaactgtgaatgatcggtgatcctggaccgtataagctgggatcagaatgaggggttatacacaactcaaaaactgaacaacagttgttctttggataactaccggttgatccaagcttcctgacagagttatccacagtagatcgcacgatctgtcagctcatttcctttaggtacaacatactagaatatttgcctacagcctcctttcggaggctgttttttta

SEQ ID NO: 11 - DNA, 582 bp, synthetic construct
  source 1..582: mol_type = other DNA
gagctgttgacagagggtcattttcacactataatgcagtgaatcccaaacagtatgttgtacctaaagggacctgcctcggtgcctgcatgacccccgccaatgatgatgacgtcaaaaggatccggataaaacatggtgattgcctcgcataacgcggtatgaaaatggattgaagcccgggccgtggattctactcaactttgtcggcttgagaaagacctgggatcctgggtattaaaaagaagatctatttatttagagatctgttctattgtgatctcttattaggatcgcactgccctgtggataacaaggatccggcttttaagatcaacaacctggaaaggatcattaactgtgaatgatcggtgatcctggaccgtataagctgggatcagaatgaggggttatacacaactcaaaaactgaacaacagttgttctttggataactaccggttgatccaagcttcctgacagagttatccacagtagatcgcacgatctgtcagctcatttcctttaggtacaacatactagaatatttgcctacagcctcctttcggaggctgttttttta

SEQ ID NO: 12 - DNA, 427 bp, synthetic construct
  source 1..427: mol_type = other DNA
gagctgttgacagagggtcattttcacactataatgccgctatagtgagtcgtagtatgttgtacctaaagggatcctgggtattaaaaagaagatctatttatttatatatatattatattattattattattaggatcgcactgccctgtggataacaaggatccggcttttaagatcaacaacctggaaaggatcattaactgtgaatgatcggtgatcctggaccgtataagctgggatcagaatgaggggttatacacagctgaggaactgaagagcagttgttctttggataactaccggttgatccaagcttcctgacagagttatccacagtagatcgcacgatctgtcagctcatttcctttaggtacaacatactagaatatttgcctacagcctcctttcggaggctgttttttta

SEQ ID NO: 13 - DNA, 37 bp, synthetic construct
  source 1..37: mol_type = other DNA
atgccgcatagtatgttgtaactaaagatctactgtg

SEQ ID NO: 14 - DNA, 47 bp, synthetic construct
  source 1..47: mol_type = other DNA
  misc_feature 11: note = dU
  misc_feature 27: note = dU
  misc_feature 41: note = dU
gtgtcggggctggcttaacagtatgttgtaactaaagtattaaaaag

SEQ ID NO: 15 - DNA, 33 bp, synthetic construct
  source 1..33: mol_type = other DNA
atgccgcattaaaaaaacagcctccgaaaggag

SEQ ID NO: 16 - DNA, 28 bp, synthetic construct
  source 1..28: mol_type = other DNA
  misc_feature 11: note = dU
  misc_feature 21: note = dU
aacgagctgttgacagagggtcattttc

SEQ ID NO: 17 - DNA, 22 bp, synthetic construct
  source 1..22: mol_type = other DNA
  misc_feature 13: note = dU
  misc_feature 20: note = dU
atcccttcagagtcccgggtag

SEQ ID NO: 18 - DNA, 31 bp, synthetic construct
  source 1..31: mol_type = other DNA
aggctgtttttttaatgcggcatcagagcag

SEQ ID NO: 19 - DNA, 37 bp, synthetic construct
  source 1..37: mol_type = other DNA
  misc_feature 9: note = dU
  misc_feature 21: note = dU
accctctgtcaacagctcgttaagccagccccgacac

SEQ ID NO: 20 - DNA, 24 bp, synthetic construct
  source 1..24: mol_type = other DNA
  misc_feature 14: note = dU
actcagactttattcaaagaccac

SEQ ID NO: 21 - DNA, 47 bp, synthetic construct
  source 1..47: mol_type = other DNA
gttaagccagccccgacacttgagatcctttttttctgcgcgtaatc

SEQ ID NO: 22 - DNA, 21 bp, synthetic construct
  source 1..21: mol_type = other DNA
ctggcgtttttccataggctc

SEQ ID NO: 23 - DNA, 19 bp, synthetic construct
  source 1..19: mol_type = other DNA
ctatgcggcatcagagcag

SEQ ID NO: 24 - DNA, 19 bp, synthetic construct
  source 1..19: mol_type = other DNA
gttaagccagccccgacac

SEQ ID NO: 25 - DNA, 76 bp, synthetic construct
  source 1..76: mol_type = other DNA
atggtgcactctcagtacaatctgctctgatgccgcatagtatgttgtaactaaagatctactgtggataactctg

SEQ ID NO: 26 - DNA, 85 bp, synthetic construct
  source 1..85: mol_type = other DNA
cgcgtcagcgggtgttggcgggtgtcggggctggcttaacagtatgttgtaactaaagtattaaaaagaagatctatttatttag

SEQ ID NO: 27 - DNA, 65 bp, synthetic construct
  source 1..65: mol_type = other DNA
cgcgtcagcgggtgttggcgggtgtcggggctggcttaacgagctgttgacagagggtcattttc

SEQ ID NO: 28 - DNA, 64 bp, synthetic construct
  source 1..64: mol_type = other DNA
atggtgcactctcagtacaatctgctctgatgccgcatagtaaaaaaacagcctccgaaaggag

SEQ ID NO: 29 - DNA, 13 bp, synthetic construct
  source 1..13: mol_type = other DNA
ggatcctgggtat

SEQ ID NO: 30 - DNA, 12 bp, synthetic construct
  source 1..12: mol_type = other DNA
cgcacgatctgt

SEQ ID NO: 31 - DNA, 20 bp, synthetic construct
  source 1..20: mol_type = other DNA
rnnnrnrkgryckynynkny

SEQ ID NO: 32 - DNA, 13 bp, synthetic construct
  source 1..13: mol_type = other DNA
tatatattatatt

SEQ ID NO: 33 - DNA, 12 bp, synthetic construct
  source 1..12: mol_type = other DNA
tattattattag

SEQ ID NO: 34 - DNA, 14 bp, synthetic construct
  source 1..14: mol_type = other DNA
gnrwgttgtaacka

SEQ ID NO: 35 - DNA, 14 bp, synthetic construct
  source 1..14: mol_type = other DNA
gkawgttgtaacka

SEQ ID NO: 36 - DNA, 14 bp, synthetic construct
  source 1..14: mol_type = other DNA
gtatgttgtaacta

SEQ ID NO: 37 - DNA, 18 bp, synthetic construct
  source 1..18: mol_type = other DNA
agtatgttgtaactaaag

SEQ ID NO: 38 - DNA, 14 bp, synthetic construct
  source 1..14: mol_type = other DNA
ggatgttgtaacta

SEQ ID NO: 39 - DNA, 14 bp, synthetic construct
  source 1..14: mol_type = other DNA
gtatgttgtaacga

SEQ ID NO: 40 - DNA, 14 bp, synthetic construct
  source 1..14: mol_type = other DNA
ggatgttgtaacta

SEQ ID NO: 41 - DNA, 14 bp, synthetic construct
  source 1..14: mol_type = other DNA
ggaagttgtaacga

SEQ ID NO: 42 - DNA, 14 bp, synthetic construct
  source 1..14: mol_type = other DNA
gtaagttgtaacga

SEQ ID NO: 43 - DNA, 14 bp, synthetic construct
  source 1..14: mol_type = other DNA
gnrwgttgtaccka

SEQ ID NO: 44 - DNA, 14 bp, synthetic construct
  source 1..14: mol_type = other DNA
gtatgttgtaccta

SEQ ID NO: 45 - DNA, 23 bp, synthetic construct
  source 1..23: mol_type = other DNA
acwrannnnnynatgtacnaaat

SEQ ID NO: 46 - DNA, 23 bp, synthetic construct
  source 1..23: mol_type = other DNA
actaattrawcyatgtactaaat

SEQ ID NO: 47 - DNA, 28 bp, synthetic construct
  source 1..28: mol_type = other DNA
actaattrawcyatgtactaaattttca

SEQ ID NO: 48 - DNA, 30 bp, synthetic construct
  source 1..30: mol_type = other DNA
gaactaattaaactatgtactaaattttca

SEQ ID NO: 49 - DNA, 30 bp, synthetic construct
  source 1..30: mol_type = other DNA
atactaattgatccatgtactaaattttca

SEQ ID NO: 50 - DNA, 13 bp, synthetic construct
  source 1..13: mol_type = other DNA
gatatgttctatt

SEQ ID NO: 51 - DNA, 13 bp, synthetic construct
  source 1..13: mol_type = other DNA
tatatattctatt

SEQ ID NO: 52 - DNA, 13 bp, synthetic construct
  source 1..13: mol_type = other DNA
ttattatattaac

SEQ ID NO: 53 - DNA, 16 bp, synthetic construct
  source 1..16: mol_type = other DNA
atatatatattctatt

SEQ ID NO: 54 - DNA, 16 bp, synthetic construct
  source 1..16: mol_type = other DNA
atatatatattatatt

SEQ ID NO: 55 - DNA, 12 bp, synthetic construct
  source 1..12: mol_type = other DNA
gattattattag

SEQ ID NO: 56 - DNA, 15 bp, synthetic construct
  source 1..15: mol_type = other DNA
gattattattaggat

SEQ ID NO: 57 - DNA, 15 bp, synthetic construct
  source 1..15: mol_type = other DNA
tattattattaggat

SEQ ID NO: 58 - DNA, 30 bp, synthetic construct
  source 1..30: mol_type = other DNA
cagcagaatatgtgatacaggatatattcc

SEQ ID NO: 59 - DNA, 23 bp, synthetic construct
  source 1..23: mol_type = other DNA
acgcaccggtgcagccttttttc

SEQ ID NO: 60 - DNA, 64 bp, synthetic construct
  source 1..64: mol_type = other DNA
tgcttcatgtggcaggagaaaaaaggctgcaccggtgcgttaaaaaaacagcctccgaaaggag

SEQ ID NO: 61 - DNA, 65 bp, synthetic construct
  source 1..65: mol_type = other DNA
gcgaggaagcggaatatatcctgtatcacatattctgctggagctgttgacagagggtcattttc

SEQ ID NO: 62 - DNA, 23 bp, synthetic construct
  source 1..23: mol_type = other DNA
cttcaaatgtagcacctgaagtc

SEQ ID NO: 63 - DNA, 23 bp, synthetic construct
  source 1..23: mol_type = other DNA
acgcaccggtgcagccttttttc

SEQ ID NO: 64 - DNA, 64 bp, synthetic construct; identical to SEQ ID NO: 60
  source 1..64: mol_type = other DNA

SEQ ID NO: 65 - DNA, 65 bp, synthetic construct
  source 1..65: mol_type = other DNA
ttatatcgtatggggctgacttcaggtgctacatttgaaggagctgttgacagagggtcattttc

SEQ ID NO: 66 - DNA, 395 bp, synthetic construct
  source 1..395: mol_type = other DNA
gtcattttcacactataatgccgctatagtgagtcgtagtatgttgtacctaaagggatcctgggtattaaaaagaagatctatttatttagagatctgttctattgtgatctcttattaggatcgcactgccctgtggataacaaggatccggcttttaagatcaacaacctggaaaggatcattaactgtgaatgatcggtgatcctggaccgtataagctgggatcagaatgaggggttatacacagctgaggaactgaagagcagttgttctttggataactaccggttgatccaagcttcctgacagagttatccacagtagatcgcacgatctgtcagctcatttcctttaggtacaacatactagaatatttgcctacagcctccttt

SEQ ID NO: 67 - DNA, 80 bp, synthetic construct
  source 1..80: mol_type = other DNA
gatctaggtgaagatcctttttgataatctcatgaccaaaatcccttaacgtgagttttcgtcattttcacactataatg

SEQ ID NO: 68 - DNA, 85 bp, synthetic construct
  source 1..85: mol_type = other DNA
tttttgtttgcaagcagcagattacgcgcagaaaaaaaggatctcaagaagatcctttgaaaaggaggctgtaggcaaatattct

SEQ ID NO: 69 - DNA, 80 bp, synthetic construct
  source 1..80: mol_type = other DNA
ggtaaatatatttatatgattatatttattatattaactatatttattgctattatcgcactgccctgtggataacaagg

SEQ ID NO: 70 - DNA, 80 bp, synthetic construct
  source 1..80: mol_type = other DNA
ttaatataataaatataatcatataaatatatttaccaattccatcattttgaaactttaggtacaacatactacgactc

SEQ ID NO: 71 - DNA, 43 bp, synthetic construct
  source 1..43: mol_type = other DNA
ttagagatatgttctattgtgattattattaggatcgcactgc

SEQ ID NO: 72 - DNA, 44 bp, synthetic construct
  source 1..44: mol_type = other DNA
cctaataataatcacaatagaacatatctctaaataaatagatc

SEQ ID NO: 73 - DNA, 45 bp, synthetic construct
  source 1..45: mol_type = other DNA
gtgaatgatctgtgatcctggactgtataagctgtgatcagaatg

SEQ ID NO: 74 - DNA, 42 bp, synthetic construct
  source 1..42: mol_type = other DNA
acagcttatacagtccaggatcacagatcattcacagttaat

SEQ ID NO: 75 - DNA, 45 bp, synthetic construct
  source 1..45: mol_type = other DNA
atttatatatatattctattgtgattattattaggatcgcactgc

SEQ ID NO: 76 - DNA, 44 bp, synthetic construct
  source 1..44: mol_type = other DNA
cctaataataatcacaatagaatatatatataaataaatagatc

SEQ ID NO: 77 - DNA, 40 bp, synthetic construct
  source 1..40: mol_type = other DNA
aggatcattaactgtgaataatctgtgatcctggactgta

SEQ ID NO: 78 - DNA, 40 bp, synthetic construct
  source 1..40: mol_type = other DNA
tacagtccaggatcacagattattcacagttaatgatcct

SEQ ID NO: 79 - DNA, 44 bp, synthetic construct
  source 1..44: mol_type = other DNA
tttatatatatattatattattattattattaggatcgcactgc

SEQ ID NO: 80 - DNA, 44 bp, synthetic construct
  source 1..44: mol_type = other DNA
cctaataataataataatataatatatatataaataaatagatc

SEQ ID NO: 81 - DNA, 50 bp, synthetic construct
  source 1..50: mol_type = other DNA
tttatttagtttttttttctattgtgatctcttattaggatcgcactgcc

SEQ ID NO: 82 - DNA, 50 bp, synthetic construct
  source 1..50: mol_type = other DNA
acaatagaaaaaaaaactaaataaatagatcttctttttaatacccagga

SEQ ID NO: 83 - DNA, 50 bp, synthetic construct
  source 1..50: mol_type = other DNA
tttatttagaaaaaaaaactattgtgatctcttattaggatcgcactgcc

SEQ ID NO: 84 - DNA, 50 bp, synthetic construct
  source 1..50: mol_type = other DNA
acaatagtttttttttctaaataaatagatcttctttttaatacccagga

SEQ ID NO: 85 - DNA, 50 bp, synthetic construct
  source 1..50: mol_type = other DNA
tattgttttttttttttttgatcgcactgccctgtggataacaaggatcc

SEQ ID NO: 86 - DNA, 50 bp, synthetic construct
  source 1..50: mol_type = other DNA
gcgatcaaaaaaaaaaaaaacaatagaacagatctctaaataaatagatc

SEQ ID NO: 87 - DNA, 50 bp, synthetic construct
  source 1..50: mol_type = other DNA
tattgtaaaaaaaaaaaaagatcgcactgccctgtggataacaaggatcc

SEQ ID NO: 88 - DNA, 50 bp, synthetic construct
  source 1..50: mol_type = other DNA
gcgatctttttttttttttacaatagaacagatctctaaataaatagatc

SEQ ID NO: 89 - DNA, 79 bp, synthetic construct
  source 1..79: mol_type = other DNA
gtattaaaaagaagatctatttatttagagatctgttctattgtgatctcttattaggatcgcactgccctgtggataa

SEQ ID NO: 90 - DNA, 79 bp, synthetic construct
  source 1..79: mol_type = other DNA
aattggtaaatatatttatatgattatatttattatattaactatatttattgctattatcgcactgccctgtggataa

SEQ ID NO: 91 - DNA, 78 bp, synthetic construct
  source 1..78: mol_type = other DNA
gtattaaaaagaagatctatttatttagagatatgttctattgtgattattattaggatcgcactgccctgtggataa

SEQ ID NO: 92 - DNA, 36 bp, synthetic construct
  source 1..36: mol_type = other DNA
agagatctgttctattgtgatctcttattaggatcg

SEQ ID NO: 93 - DNA, 35 bp, synthetic construct
  source 1..35: mol_type = other DNA
agagatatgttctattgtgattattattaggatcg

SEQ ID NO: 94 - DNA, 35 bp, synthetic construct
  source 1..35: mol_type = other DNA
atatatatattctattgtgattattattaggatcg

SEQ ID NO: 95 - DNA, 38 bp, synthetic construct
  source 1..38: mol_type = other DNA
tcggtgatcctggaccgtataagctgggatcagaatga

SEQ ID NO: 96 - DNA, 38 bp, synthetic construct; identical to SEQ ID NO: 95
  source 1..38: mol_type = other DNA

SEQ ID NO: 97 - DNA, 38 bp, synthetic construct
  source 1..38: mol_type = other DNA
tctgtgatcctggactgtataagctgtgatcagaatga

SEQ ID NO: 98 - DNA, 36 bp, synthetic construct; identical to SEQ ID NO: 92
  source 1..36: mol_type = other DNA

SEQ ID NO: 99 - DNA, 35 bp, synthetic construct; identical to SEQ ID NO: 94
  source 1..35: mol_type = other DNA

SEQ ID NO: 100 - DNA, 35 bp, synthetic construct
  source 1..35: mol_type = other DNA
atatatatattatattgtgattattattaggatcg

SEQ ID NO: 101 - DNA, 49 bp, synthetic construct
  source 1..49: mol_type = other DNA
actgtgaatgatcggtgatcctggaccgtataagctgggatcagaatga

SEQ ID NO: 102 - DNA, 49 bp, synthetic construct
  source 1..49: mol_type = other DNA
actgtgaatgatctgtgatcctggactgtataagctgtgatcagaatga

SEQ ID NO: 103 - DNA, 49 bp, synthetic construct
  source 1..49: mol_type = other DNA
actgtgaataatctgtgatcctggactgtataagctgtgatcagaatga

SEQ ID NO: 104 - DNA, 36 bp, synthetic construct; identical to SEQ ID NO: 92
  source 1..36: mol_type = other DNA

SEQ ID NO: 105 - DNA, 36 bp, synthetic construct
  source 1..36: mol_type = other DNA
agtttttttttctattgtgatctcttattaggatcg

SEQ ID NO: 106 - DNA, 36 bp, synthetic construct
  source 1..36: mol_type = other DNA
agaaaaaaaaactattgtgatctcttattaggatcg

SEQ ID NO: 107 - DNA, 36 bp, synthetic construct
  source 1..36: mol_type = other DNA
agagatctgttctattgttttttttttttttgatcg

SEQ ID NO: 108 - DNA, 36 bp, synthetic construct
  source 1..36: mol_type = other DNA
agagatctgttctattgtaaaaaaaaaaaaagatcg

SEQ ID NO: 109 - DNA, 583 bp, synthetic construct
  source 1..583: mol_type = other DNA
gagctgttgacagagggtcattttcacactataatgccgctatagtgagtcgtagtatgttgtacctaaagggacctgtttttgatgccatcagaaaacgcgtcagcgccgctctgaggcaataaacagaatcaggcataaaatcagccgcacagattttttaaaacgcgccacgggatttttaaaccggtatttaacggtgtatgaatcccgttttatcttcctttggatcctgggtattaaaaagaagatctatttatttatatatatattatattattattattattaggatcgcactgccctgtggataacaaggatccggcttttaagatcaacaacctggaaaggatcattaactgtgaatgatcggtgatcctggaccgtataagctgggatcagaatgaggggttatacacagctgaggaactgaagagcagttgttctttggataactaccggttgatccaagcttcctgacagagttatccacagtagatcgcacgatctgtcagctcatttcctttaggtacaacatactagaatatttgcctacagcctcctttcggaggctgttttttta

SEQ ID NO: 110 - DNA, 13 bp, synthetic construct
  source 1..13: mol_type = other DNA
gatctnttntttt

SEQ ID NO: 111 - DNA, 44 bp, synthetic construct
  source 1..44: mol_type = other DNA
gatctatttatttagagatctgttctattgtgatctcttattag

SEQ ID NO: 112 - DNA, 13 bp, synthetic construct
  source 1..13: mol_type = other DNA
gatctatttattt

SEQ ID NO: 113 - DNA, 13 bp, synthetic construct
  source 1..13: mol_type = other DNA
gatctgttctatt

SEQ ID NO: 114 - DNA, 13 bp, synthetic construct
  source 1..13: mol_type = other DNA
gatctcttattag

SEQ ID NO: 115 - DNA, 16 bp, synthetic construct
  source 1..16: mol_type = other DNA
gtattattattaggat

SEQ ID NO: 116 - DNA, 16 bp, synthetic construct
  source 1..16: mol_type = other DNA
gtatatatattaggat